European Patent Application EP 4 578 449 A1, published July 2, 2025. Title: PHARMACEUTICAL COMBINATION OF FAK INHIBITOR AND MICROTUBULE INHIBITOR AND USE THEREOF. Applicant: INXMED (NANJING) CO., LTD. The sequence listing filed with the application follows.

SEQUENCE LISTING (4 sequences)

SEQ ID NO: 1 - RNA, 21 nt, synthetic construct
  source 1..21: mol_type = other RNA; note = forward strand
cctgtatgcctatcagctttt

SEQ ID NO: 2 - RNA, 21 nt, synthetic construct
  source 1..21: mol_type = other RNA; note = reverse strand
aagctgataggcatacaggtt

SEQ ID NO: 3 - RNA, 21 nt, synthetic construct
  source 1..21: mol_type = other RNA; note = forward strand
cctgtatgcctatcagctttt

SEQ ID NO: 4 - RNA, 21 nt, synthetic construct
  source 1..21: mol_type = other RNA; note = reverse strand
aagctgataggcatacaggtt